European Patent Application EP 4 215 619 A1, published July 26, 2023. Title: METHODS FOR SENSITIVE AND ACCURATE PARALLEL QUANTIFICATION OF NUCLEIC ACIDS. Applicant: Genomill Health Oy. The sequence listing filed with the application follows.

SEQUENCE LISTING (28 sequences)

SEQ ID NO: 1 - DNA, 31 bp, Artificial Sequence
  random sequence
ggggcccgccgtcgatcggagccgttaggat

SEQ ID NO: 2 - DNA, 31 bp, Artificial Sequence
  random sequence - just for illustration
ttaaggtgccgtcgatcggagccgacgtacg

SEQ ID NO: 3 - DNA, 31 bp, Artificial Sequence; identical to SEQ ID NO: 2
  random sequence - just for illustration

SEQ ID NO: 4 - DNA, 31 bp, Artificial Sequence
  random sequence - just for illustration
tataatagaggtcgtgcagtcacgacccggt

SEQ ID NO: 5 - DNA, 31 bp, Artificial Sequence
  random sequence - just for illustration
accaggtgccgtcgatcggagccgacccggt

SEQ ID NO: 6 - DNA, 31 bp, Artificial Sequence
  random sequence - just for illustration
gggccgggaggtcgtgcagtcacgttaggat

SEQ ID NO: 7 - DNA, 31 bp, Artificial Sequence
  random sequence - just for illustration
tccaggtgagtcgatccgtcacgtacgtacg

SEQ ID NO: 8 - DNA, 31 bp, Artificial Sequence
  random sequence - just for illustration
aaaattttagcgtacgtcgtacgtttaggat

SEQ ID NO: 9 - DNA, 31 bp, Artificial Sequence; identical to SEQ ID NO: 4
  random sequence - just for illustration

SEQ ID NO: 10 - DNA, 31 bp, Artificial Sequence
  random sequence - just for illustration
aggaccttgagtcgatccgcacgtacccggt

SEQ ID NO: 11 - DNA, 31 bp, Artificial Sequence
  random sequence - just for illustration
agcgaccgaggtcgtgcagtcacgacgtacg

SEQ ID NO: 12 - DNA, 31 bp, Artificial Sequence; identical to SEQ ID NO: 4
  random sequence - just for illustration

SEQ ID NO: 13 - DNA, 31 bp, Artificial Sequence
  random sequence - just for illustration
ggaaaaagccgtcgatcggagccgttaggat

SEQ ID NO: 14 - DNA, 31 bp, Artificial Sequence
  random sequence - just for illustration
atatacagaggtcgtgcagtcacgttaggat

SEQ ID NO: 15 - DNA, 31 bp, Artificial Sequence
  random sequence - just for illustration
gagagccgaggtcgtgcagtcacgacccggt

SEQ ID NO: 16 - DNA, 31 bp, Artificial Sequence
  random sequence - just for illustration
cgcacgcgaggtcgtgcagtcacgacgtacg

SEQ ID NO: 17 - DNA, 31 bp, Artificial Sequence
  random sequence - just for illustration
attacaagccgtcgatcggagccgacccggt

SEQ ID NO: 18 - DNA, 31 bp, Artificial Sequence; identical to SEQ ID NO: 4
  random sequence - just for illustration

SEQ ID NO: 19 - DNA, 31 bp, Artificial Sequence
  random sequence - just for illustration
gggcaattagcgtacgtcgtacgtacgtacg

SEQ ID NO: 20 - DNA, 31 bp, Artificial Sequence
  random sequence - just for illustration
tatgcgagccgtcgatcggagccgacgtacg

SEQ ID NO: 21 - DNA, 31 bp, Artificial Sequence; identical to SEQ ID NO: 10
  random sequence - just for illustration

SEQ ID NO: 22 - DNA, 31 bp, Artificial Sequence; identical to SEQ ID NO: 17
  random sequence - just for illustration

SEQ ID NO: 23 - DNA, 31 bp, Artificial Sequence
  random sequence - just for illustration
gaagaattagcgtacgtcgtacgtttaggat

SEQ ID NO: 24 - DNA, 31 bp, Artificial Sequence; identical to SEQ ID NO: 19
  random sequence - just for illustration

SEQ ID NO: 25 - DNA, 31 bp, Artificial Sequence; identical to SEQ ID NO: 19
  random sequence - just for illustration

SEQ ID NO: 26 - DNA, 31 bp, Artificial Sequence
  random sequence - just for illustration
gagcacttagcgtacgtcgtacgtacccggt

SEQ ID NO: 27 - DNA, 31 bp, Artificial Sequence
  random sequence - just for illustration
aaaggggcgagtcgatccgcacgtttaggat

SEQ ID NO: 28 - DNA, 31 bp, Artificial Sequence
  random sequence - just for illustration
agcgcgcgccgtcgatcggagccgttaggat